European Patent Application EP 4 534 682 A1, published April 9, 2025. Title: 나노입자-올리고T 결합체를 기반으로 하는 메신저 RNA 운반 체. Applicant: NES BIOTECHNOLOGY. The sequence listing filed with the application follows.

SEQUENCE LISTING (5 sequences)

SEQ ID NO: 1 - DNA, 28 bp, synthetic construct
  source 1..28: mol_type = other DNA
tttttttttttttttttttttttttttt

SEQ ID NO: 2 - DNA, 20 bp, synthetic construct
  source 1..20: mol_type = other DNA
aaaaaaaaaaaaaaaaaaaa

SEQ ID NO: 3 - DNA, 837 bp, synthetic construct
  source 1..837: mol_type = other DNA
taatacgactcactataaggcgctagcagagccgagatgccgccaccatggtgagcaagggcgaggagctgttcaccggggtggtgcccatcctggtcgagctggacggcgacgtaaacggccacaagttcagcgtgtccggcgagggcgagggcgatgccacctacggcaagctgaccctgaagttcatctgcaccaccggcaagctgcccgtgccctggcccaccctcgtgaccaccctgacctacggcgtgcagtgcttcagccgctaccccgaccacatgaagcagcacgacttcttcaagtccgccatgcccgaaggctacgtccaggagcgcaccatcttcttcaaggacgacggcaactacaagacccgcgccgaggtgaagttcgagggcgacaccctggtgaaccgcatcgagctgaagggcatcgacttcaaggaggacggcaacatcctggggcacaagctggagtacaactacaacagccacaacgtctatatcatggccgacaagcagaagaacggcatcaaggtgaacttcaagatccgccacaacatcgaggacggcagcgtgcagctcgccgaccactaccagcagaacacccccatcggcgacggccccgtgctgctgcccgacaaccactacctgagcacccagtccgccctgagcaaagaccccaacgagaagcgcgatcacatggtcctgctggagttcgtgaccgccgccgggatcactctcggcatggacgagctgtacaagtaaaaaaaaaaaaaaaaaaaaaaaaaaaaaaaaaaaaaaaaaaaaaaaaaaaaaaaaaaaaaaaaaaaaaaaa

SEQ ID NO: 4 - DNA, 837 bp, synthetic construct
  source 1..837: mol_type = other DNA
taatacgactcactataaggcgctagcagagccgagatgccgccaccatgttcgtgttcctggtgctgctgcctctggtgtccagccagtgtgtgagggtccaaccaacagagagcattgtgaggtttccaaacatcaccaacctgtgtccatttggagaggtgttcaatgccaccaggtttgcctctgtctatgcctggaacaggaagaggattagcaactgtgtggctgactactctgtgctctacaactctgcctccttcagcaccttcaagtgttatggagtgagcccaaccaaactgaatgacctgtgtttcaccaatgtctatgctgactcctttgtgattaggggagatgaggtgagacagattgcccctggacaaacaggcaagattgctgactacaactacaaactgcctgatgacttcacaggctgtgtgattgcctggaacagcaacaacctggacagcaaggtgggaggcaactacaactaccggtacagactgttcaggaagagcaacctgaaaccatttgagagggacatcagcacagagatttaccaggctggcagcaagccatgtaatggagtggagggcttcaactgttactttccactccaatcctatggcttccaaccaaccaatggagtgggctaccaaccatacagggtggtggtgctgtcctttgaactgctccatgcccctgccacagtgtgtggaccaaagaagagcaccaacctggtgaagaacaagtgtgtgaacttctgaaaaaaaaaaaaaaaaaaaaaaaaaaaaaaaaaaaaaaaaaaaaaaaaaaaaaaaaaaaaaaaaaaaaaaa

SEQ ID NO: 5 - DNA, 15 bp, synthetic construct
  source 1..15: mol_type = other DNA
taatacgactcacta